European Patent Application EP 4 357 454 A2, published April 24, 2024. Title: TRANSFECTED T-CELLS AND T-CELL RECEPTORS FOR USE IN IMMUNOTHERAPY AGAINST CANCERS. Applicant: Immatics Biotechnologies GmbH. Application WO PCT/EP2017 /056260, filed March 16, 2017. The sequence listing filed with the application follows.

SEQUENCE LISTING (101 sequences)

SEQ ID NO: 1 - protein, 9 aa, Homo sapiens
KVLEHVVRV

SEQ ID NO: 2 - protein, 9 aa, Homo sapiens
KVLEHVVRL

SEQ ID NO: 3 - protein, 9 aa, Homo sapiens
KVLEHVVRA

SEQ ID NO: 4 - protein, 9 aa, Homo sapiens
KVLEHVVRI

SEQ ID NO: 5 - protein, 9 aa, Homo sapiens
KLLEHVVRV

SEQ ID NO: 6 - protein, 9 aa, Homo sapiens
KLLEHVVRL

SEQ ID NO: 7 - protein, 9 aa, Homo sapiens
KLLEHVVRA

SEQ ID NO: 8 - protein, 9 aa, Homo sapiens
KLLEHVVRI

SEQ ID NO: 9 - protein, 9 aa, Homo sapiens
KALEHVVRV

SEQ ID NO: 10 - protein, 9 aa, Homo sapiens
KALEHVVRL

SEQ ID NO: 11 - protein, 9 aa, Homo sapiens
KALEHVVRA

SEQ ID NO: 12 - protein, 9 aa, Homo sapiens
KALEHVVRI

SEQ ID NO: 13 - protein, 9 aa, Homo sapiens
YLLEHVVRV

SEQ ID NO: 14 - protein, 9 aa, Homo sapiens
YLLEHVVRL

SEQ ID NO: 15 - protein, 9 aa, Homo sapiens
YLLEHVVRA

SEQ ID NO: 16 - protein, 9 aa, Homo sapiens
YLLEHVVRI

SEQ ID NO: 17 - protein, 9 aa, Homo sapiens
YALEHVVRV

SEQ ID NO: 18 - protein, 9 aa, Homo sapiens
YALEHVVRL

SEQ ID NO: 19 - protein, 9 aa, Homo sapiens
YALEHVVRA

SEQ ID NO: 20 - protein, 9 aa, Homo sapiens
YALEHVVRI

SEQ ID NO: 21 - protein, 9 aa, Homo sapiens
YVLEHVVRV

SEQ ID NO: 22 - protein, 9 aa, Homo sapiens
YVLEHVVRL

SEQ ID NO: 23 - protein, 9 aa, Homo sapiens
YVLEHVVRA

SEQ ID NO: 24 - protein, 9 aa, Homo sapiens
YVLEHVVRI

SEQ ID NO: 25 - protein, 9 aa, Homo sapiens
  SITE 1: note = misc_feature - Xaa can be Lys or Tyr
  SITE 2: note = misc_feature - Xaa can be Val, Leu or Ala
  SITE 9: note = misc_feature - Xaa can be Val, Leu, Ala or Ile
XXLEHVVRX

SEQ ID NO: 26 - DNA, 36 bp, Homo sapiens
  source 1..36: mol_type = other DNA
ggaattccatatgagtcaacaaggagaagaagatcc

SEQ ID NO: 27 - DNA, 36 bp, Homo sapiens
  source 1..36: mol_type = other DNA
ttgtcagtcgacttagagtctctcagctggtacacg

SEQ ID NO: 28 - DNA, 36 bp, Homo sapiens
  source 1..36: mol_type = other DNA
tctctcatatggatggtggaattactcaatccccaa

SEQ ID NO: 29 - DNA, 32 bp, Homo sapiens
  source 1..32: mol_type = other DNA
tagaaaccggtggccaggcacaccagtgtggc

SEQ ID NO: 30 - protein, 9 aa, Homo sapiens
AVLEHVVRV

SEQ ID NO: 31 - protein, 9 aa, Homo sapiens
KALEHVVRV

SEQ ID NO: 32 - protein, 9 aa, Homo sapiens
KVAEHVVRV

SEQ ID NO: 33 - protein, 9 aa, Homo sapiens
KVLAHVVRV

SEQ ID NO: 34 - protein, 9 aa, Homo sapiens
KVLEAVVRV

SEQ ID NO: 35 - protein, 9 aa, Homo sapiens
KVLEHAVRV

SEQ ID NO: 36 - protein, 9 aa, Homo sapiens
KVLEHVARV

SEQ ID NO: 37 - protein, 9 aa, Homo sapiens
KVLEHVVAV

SEQ ID NO: 38 - protein, 9 aa, Homo sapiens
KVLEHVVRA

SEQ ID NO: 39 - protein, 274 aa, Homo sapiens
MEKMLECAFIVLWLQLGWLSGEDQVTQSPEALRLQEGESSSLNCSYTVSGLRGLFWYRQDPGKGPEFLFTLYSAGEEKEKERLKATLTKKESFLHITAPKPEDSATYLCAVQGENSGYSTLTFGKGTMLLVSPDIQNPDPAVYQLRDSKSSDKSVCLFTDFDSQTNVSQSKDSDVYITDKTVLDMRSMDFKSNSAVAWSNKSDFACANAFNNSIIPEDTFFPSPESSCDVKLVEKSFETDTNLNFQNLSVIGFRILLLKVAGFNLLMTLRLWSS

SEQ ID NO: 40 - protein, 21 aa, Homo sapiens
MEKMLECAFIVLWLQLGWLSG

SEQ ID NO: 41 - protein, 112 aa, Homo sapiens
MEKMLECAFIVLWLQLGWLSGEDQVTQSPEALRLQEGESSSLNCSYTVSGLRGLFWYRQDPGKGPEFLFTLYSAGEEKEKERLKATLTKKESFLHITAPKPEDSATYLCAVQ

SEQ ID NO: 42 - protein, 6 aa, Homo sapiens
VSGLRG

SEQ ID NO: 43 - skipped

SEQ ID NO: 44 - protein, 15 aa, Homo sapiens
CAVQGENSGYSTLTF

SEQ ID NO: 45 - protein, 19 aa, Homo sapiens
NSGYSTLTFGKGTMLLVSP

SEQ ID NO: 46 - protein, 141 aa, Homo sapiens
DIQNPDPAVYQLRDSKSSDKSVCLFTDFDSQTNVSQSKDSDVYITDKTVLDMRSMDFKSNSAVAWSNKSDFACANAFNNSIIPEDTFFPSPESSCDVKLVEKSFETDTNLNFQNLSVIGFRILLLKVAGFNLLMTLRLWSS

SEQ ID NO: 47 - protein, 314 aa, Homo sapiens
MGPQLLGYVVLCLLGAGPLEAQVTQNPRYLITVTGKKLTVTCSQNMNHEYMSWYRQDPGLGLRQIYYSMNVEVTDKGDVPEGYKVSRKEKRNFPLILESPSPNQTSLYFCASSLGPGLAAYNEQFFGPGTRLTVLEDLKNVFPPEVAVFEPSEAEISHTQKATLVCLATGFYPDHVELSWWVNGKEVHSGVSTDPQPLKEQPALNDSRYCLSSRLRVSATFWQNPRNHFRCQVQFYGLSENDEWTQDRAKPVTQIVSAEAWGRADCGFTSESYQQGVLSATILYEILLGKATLYAVLVSALVLMAMVKRKDSRG

SEQ ID NO: 48 - protein, 19 aa, Homo sapiens
MGPQLLGYVVLCLLGAGPL

SEQ ID NO: 49 - protein, 114 aa, Homo sapiens
MGPQLLGYVVLCLLGAGPLEAQVTQNPRYLITVTGKKLTVTCSQNMNHEYMSWYRQDPGLGLRQIYYSMNVEVTDKGDVPEGYKVSRKEKRNFPLILESPSPNQTSLYFCASSL

SEQ ID NO: 50 - protein, 5 aa, Homo sapiens
MNHEY

SEQ ID NO: 51 - protein, 6 aa, Homo sapiens
SMNVEV

SEQ ID NO: 52 - protein, 16 aa, Homo sapiens
CASSLGPGLAAYNEQF

SEQ ID NO: 53 - protein, 15 aa, Homo sapiens
YNEQFFGPGTRLTVL

SEQ ID NO: 54 - protein, 179 aa, Homo sapiens
EDLKNVFPPEVAVFEPSEAEISHTQKATLVCLATGFYPDHVELSWWVNGKEVHSGVSTDPQPLKEQPALNDSRYCLSSRLRVSATFWQNPRNHFRCQVQFYGLSENDEWTQDRAKPVTQIVSAEAWGRADCGFTSESYQQGVLSATILYEILLGKATLYAVLVSALVLMAMVKRKDSRG

SEQ ID NO: 55 - protein, 272 aa, Homo sapiens
MKTFAGFSFLFLWLQLDCMSRGEDVEQSLFLSVREGDSSVINCTYTDSSSTYLYWYKQEPGAGLQLLTYIFSNMDMKQDQRLTVLLNKKDKHLSLRIADTQTGDSAIYFCAEYSSASKIIFGSGTRLSIRPNIQNPDPAVYQLRDSKSSDKSVCLFTDFDSQTNVSQSKDSDVYITDKTVLDMRSMDFKSNSAVAWSNKSDFACANAFNNSIIPEDTFFPSPESSCDVKLVEKSFETDTNLNFQNLSVIGFRILLLKVAGFNLLMTLRLWSS

SEQ ID NO: 56 - protein, 21 aa, Homo sapiens
MKTFAGFSFLFLWLQLDCMSR

SEQ ID NO: 57 - protein, 112 aa, Homo sapiens
MKTFAGFSFLFLWLQLDCMSRGEDVEQSLFLSVREGDSSVINCTYTDSSSTYLYWYKQEPGAGLQLLTYIFSNMDMKQDQRLTVLLNKKDKHLSLRIADTQTGDSAIYFCAE

SEQ ID NO: 58 - protein, 6 aa, Homo sapiens
DSSSTY

SEQ ID NO: 59 - skipped

SEQ ID NO: 60 - protein, 12 aa, Homo sapiens
CAEYSSASKIIF

SEQ ID NO: 61 - protein, 19 aa, Homo sapiens
YSSASKIIFGSGTRLSIRP

SEQ ID NO: 62 - protein, 141 aa, Homo sapiens
NIQNPDPAVYQLRDSKSSDKSVCLFTDFDSQTNVSQSKDSDVYITDKTVLDMRSMDFKSNSAVAWSNKSDFACANAFNNSIIPEDTFFPSPESSCDVKLVEKSFETDTNLNFQNLSVIGFRILLLKVAGFNLLMTLRLWSS

SEQ ID NO: 63 - protein, 310 aa, Homo sapiens
MGSWTLCCVSLCILVAKHTDAGVIQSPRHEVTEMGQEVTLRCKPISGHDYLFWYRQTMMRGLELLIYFNNNVPIDDSGMPEDRFSAKMPNASFSTLKIQPSEPRDSAVYFCASRANTGELFFGEGSRLTVLEDLKNVFPPEVAVFEPSEAEISHTQKATLVCLATGFYPDHVELSWWVNGKEVHSGVSTDPQPLKEQPALNDSRYCLSSRLRVSATFWQNPRNHFRCQVQFYGLSENDEWTQDRAKPVTQIVSAEAWGRADCGFTSESYQQGVLSATILYEILLGKATLYAVLVSALVLMAMVKRKDSRG

SEQ ID NO: 64 - protein, 19 aa, Homo sapiens
MGSWTLCCVSLCILVAKHT

SEQ ID NO: 65 - protein, 113 aa, Homo sapiens
MGSWTLCCVSLCILVAKHTDAGVIQSPRHEVTEMGQEVTLRCKPISGHDYLFWYRQTMMRGLELLIYFNNNVPIDDSGMPEDRFSAKMPNASFSTLKIQPSEPRDSAVYFCAS

SEQ ID NO: 66 - protein, 5 aa, Homo sapiens
SGHDY

SEQ ID NO: 67 - protein, 6 aa, Homo sapiens
FNNNVP

SEQ ID NO: 68 - protein, 12 aa, Homo sapiens
CASRANTGELFF

SEQ ID NO: 69 - protein, 16 aa, Homo sapiens
NTGELFFGEGSRLTVL

SEQ ID NO: 70 - protein, 179 aa, Homo sapiens; identical to SEQ ID NO: 54

SEQ ID NO: 71 - protein, 277 aa, Homo sapiens
MLTASLLRAVIASICVVSSMAQKVTQAQTEISVVEKEDVTLDCVYETRDTTYYLFWYKQPPSGELVFLIRRNSFDEQNEISGRYSWNFQKSTSSFNFTITASQVVDSAVYFCALSEGNSGNTPLVFGKGTRLSVIANIQNPDPAVYQLRDSKSSDKSVCLFTDFDSQTNVSQSKDSDVYITDKTVLDMRSMDFKSNSAVAWSNKSDFACANAFNNSIIPEDTFFPSPESSCDVKLVEKSFETDTNLNFQNLSVIGFRILLLKVAGFNLLMTLRLWSS

SEQ ID NO: 72 - protein, 20 aa, Homo sapiens
MLTASLLRAVIASICVVSSM

SEQ ID NO: 73 - protein, 116 aa, Homo sapiens
MLTASLLRAVIASICVVSSMAQKVTQAQTEISVVEKEDVTLDCVYETRDTTYYLFWYKQPPSGELVFLIRRNSFDEQNEISGRYSWNFQKSTSSFNFTITASQVVDSAVYFCALSE

SEQ ID NO: 74 - protein, 7 aa, Homo sapiens
TRDTTYY

SEQ ID NO: 75 - protein, 4 aa, Homo sapiens
RNSF

SEQ ID NO: 76 - protein, 15 aa, Homo sapiens
CALSEGNSGNTPLVF

SEQ ID NO: 77 - protein, 19 aa, Homo sapiens
NSGNTPLVFGKGTRLSVIA

SEQ ID NO: 78 - protein, 141 aa, Homo sapiens; identical to SEQ ID NO: 62

SEQ ID NO: 79 - protein, 313 aa, Homo sapiens
MGIRLLCRVAFCFLAVGLVDVKVTQSSRYLVKRTGEKVFLECVQDMDHENMFWYRQDPGLGLRLIYFSYDVKMKEKGDIPEGYSVSREKKERFSLILESASTNQTSMYLCASSLSSGSHQETQYFGPGTRLLVLEDLKNVFPPEVAVFEPSEAEISHTQKATLVCLATGFYPDHVELSWWVNGKEVHSGVSTDPQPLKEQPALNDSRYCLSSRLRVSATFWQNPRNHFRCQVQFYGLSENDEWTQDRAKPVTQIVSAEAWGRADCGFTSESYQQGVLSATILYEILLGKATLYAVLVSALVLMAMVKRKDSRG

SEQ ID NO: 80 - protein, 19 aa, Homo sapiens
MGIRLLCRVAFCFLAVGLV

SEQ ID NO: 81 - protein, 114 aa, Homo sapiens
MGIRLLCRVAFCFLAVGLVDVKVTQSSRYLVKRTGEKVFLECVQDMDHENMFWYRQDPGLGLRLIYFSYDVKMKEKGDIPEGYSVSREKKERFSLILESASTNQTSMYLCASSL

SEQ ID NO: 82 - protein, 5 aa, Homo sapiens
MDHEN

SEQ ID NO: 83 - protein, 6 aa, Homo sapiens
SYDVKM

SEQ ID NO: 84 - protein, 16 aa, Homo sapiens
CASSLSSGSHQETQYF

SEQ ID NO: 85 - protein, 15 aa, Homo sapiens
QETQYFGPGTRLLVL

SEQ ID NO: 86 - protein, 179 aa, Homo sapiens; identical to SEQ ID NO: 54

SEQ ID NO: 87 - protein, 20 aa, Homo sapiens
VIGFRILLLKVAGFNLLMTL

SEQ ID NO: 88 - protein, 23 aa, Homo sapiens
TILYEILLGKATLYAVLVSALVL

SEQ ID NO: 89 - protein, 274 aa, Homo sapiens
METLLGLLILWLQLQWVSSKQEVTQIPAALSVPEGENLVLNCSFTDSAIYNLQWFRQDPGKGLTSLLLIQSSQREQTSGRLNASLDKSSGRSTLYIAASQPGDSATYLCAVRPTSGGSYIPTFGRGTSLIVHPYIQNPDPAVYQLRDSKSSDKSVCLFTDFDSQTNVSQSKDSDVYITDKTVLDMRSMDFKSNSAVAWSNKSDFACANAFNNSIIPEDTFFPSPESSCDVKLVEKSFETDTNLNFQNLSVIGFRILLLKVAGFNLLMTLRLWSS

SEQ ID NO: 90 - protein, 311 aa, Homo sapiens
MSIGLLCCAALSLLWAGPVNAGVTQTPKFQVLKTGQSMTLQCAQDMNHEYMSWYRQDPGMGLRLIHYSVGAGITDQGEVPNGYNVSRSTTEDFPLRLLSAAPSQTSVYFCASSYVGNTGELFFGEGSRLTVLEDLKNVFPPEVAVFEPSEAEISHTQKATLVCLATGFYPDHVELSWWVNGKEVHSGVSTDPQPLKEQPALNDSRYCLSSRLRVSATFWQNPRNHFRCQVQFYGLSENDEWTQDRAKPVTQIVSAEAWGRADCGFTSESYQQGVLSATILYEILLGKATLYAVLVSALVLMAMVKRKDSRG

SEQ ID NO: 91 - protein, 9 aa, Homo sapiens
FLLETVVRV

SEQ ID NO: 92 - protein, 9 aa, Homo sapiens
ILDEHVQRV

SEQ ID NO: 93 - protein, 9 aa, Homo sapiens
IVMEHVVFL

SEQ ID NO: 94 - protein, 9 aa, Homo sapiens
KILEDVVGV

SEQ ID NO: 95 - protein, 9 aa, Homo sapiens
KLLDLQVRV

SEQ ID NO: 96 - protein, 9 aa, Homo sapiens
KVLDKVFRA

SEQ ID NO: 97 - protein, 9 aa, Homo sapiens
KVLEILHRV

SEQ ID NO: 98 - protein, 9 aa, Homo sapiens
KVLERVNAV

SEQ ID NO: 99 - protein, 9 aa, Homo sapiens
KVLETLVTV

SEQ ID NO: 100 - protein, 9 aa, Homo sapiens
KVLGIVVGV

SEQ ID NO: 101 - protein, 9 aa, Homo sapiens
SLLMWITQV